European Patent Application EP 4 410 843 A1, published August 7, 2024. Title: Recombinant fusion protein derived from HR region of S2 protein of SARS-COV-2 and application of recombinant fusion protein. Applicant: 上海神州科冠生物医药有限公司. The sequence listing filed with the application follows.

SEQUENCE LISTING (30 sequences)

SEQ ID NO: 1 - protein, 77 aa, synthetic construct
  source 1..77: note = Amino acid sequence of HR1
TQNVLYENQKLIANQFNSAIGKIQDSLSSTASALGKLQDVVNQNAQALNTLVKQLSSNFGAISSVLNDILSRLDKVE

SEQ ID NO: 2 - protein, 44 aa, synthetic construct
  source 1..44: note = Amino acid sequence of HR2
DVDLGDISGINASVVNIQKEIDRLNEVAKNLNESLIDLQELGKY

SEQ ID NO: 3 - protein, 5 aa, synthetic construct
  source 1..5: note = Linker1
GGSGG

SEQ ID NO: 4 - protein, 6 aa, synthetic construct
  source 1..6: note = Linker2
SGGRGG

SEQ ID NO: 5 - protein, 209 aa, synthetic construct
  source 1..209: note = Amino acid sequence of HR121
TQNVLYENQKLIANQFNSAIGKIQDSLSSTASALGKLQDVVNQNAQALNTLVKQLSSNFGAISSVLNDILSRLDKVEGGSGGDVDLGDISGINASVVNIQKEIDRLNEVAKNLNESLIDLQELGKYSGGRGGTQNVLYENQKLIANQFNSAIGKIQDSLSSTASALGKLQDVVNQNAQALNTLVKQLSSNFGAISSVLNDILSRLDKVE

SEQ ID NO: 6 - protein, 176 aa, synthetic construct
  source 1..176: note = Amino acid sequence of HR212
DVDLGDISGINASVVNIQKEIDRLNEVAKNLNESLIDLQELGKYSGGRGGTQNVLYENQKLIANQFNSAIGKIQDSLSSTASALGKLQDVVNQNAQALNTLVKQLSSNFGAISSVLNDILSRLDKVEGGSGGDVDLGDISGINASVVNIQKEIDRLNEVAKNLNESLIDLQELGKY

SEQ ID NO: 7 - DNA, 630 bp, synthetic construct
  source 1..630: mol_type = other DNA; note = The nucleotide sequence encoding HR121
acacagaatgttctctatgagaaccaaaaattgattgccaaccaatttaatagtgctattggcaaaattcaagactcactttcttccacagcaagtgcacttggaaaacttcaagatgtggtcaaccaaaatgcacaagctttaaacacgcttgttaaacaacttagctccaattttggtgcaatttcaagtgttttaaatgatatcctttcacgtcttgacaaagttgagggaggaagcggaggagatgttgatttaggtgacatctctggcattaatgcttcagttgtaaacattcaaaaagaaattgaccgcctcaatgaggttgccaagaatttaaatgaatctctcatcgatctccaagaacttggaaagtatagcggaggaagaggaggaacacagaatgttctctatgagaaccaaaaattgattgccaaccaatttaatagtgctattggcaaaattcaagactcactttcttccacagcaagtgcacttggaaaacttcaagatgtggtcaaccaaaatgcacaagctttaaacacgcttgttaaacaacttagctccaattttggtgcaatttcaagtgttttaaatgatatcctttcacgtcttgacaaagttgagtaa

SEQ ID NO: 8 - DNA, 531 bp, synthetic construct
  source 1..531: mol_type = other DNA; note = The nucleotide sequence encoding HR212
gatgttgatttaggtgacatctctggcattaatgcttcagttgtaaacattcaaaaagaaattgaccgcctcaatgaggttgccaagaatttaaatgaatctctcatcgatctccaagaacttggaaagtatagcggaggaagaggaggaacacagaatgttctctatgagaaccaaaaattgattgccaaccaatttaatagtgctattggcaaaattcaagactcactttcttccacagcaagtgcacttggaaaacttcaagatgtggtcaaccaaaatgcacaagctttaaacacgcttgttaaacaacttagctccaattttggtgcaatttcaagtgttttaaatgatatcctttcacgtcttgacaaagttgagggaggaagcggaggagatgttgatttaggtgacatctctggcattaatgcttcagttgtaaacattcaaaaagaaattgaccgcctcaatgaggttgccaagaatttaaatgaatctctcatcgatctccaagaacttggaaagtattaa

SEQ ID NO: 9 - DNA, 231 bp, synthetic construct
  source 1..231: mol_type = other DNA; note = The nucleotide sequence encoding HR1
acacagaatgttctctatgagaaccaaaaattgattgccaaccaatttaatagtgctattggcaaaattcaagactcactttcttccacagcaagtgcacttggaaaacttcaagatgtggtcaaccaaaatgcacaagctttaaacacgcttgttaaacaacttagctccaattttggtgcaatttcaagtgttttaaatgatatcctttcacgtcttgacaaagttgag

SEQ ID NO: 10 - DNA, 132 bp, synthetic construct
  source 1..132: mol_type = other DNA; note = The nucleotide sequence encoding HR2
gatgttgatttaggtgacatctctggcattaatgcttcagttgtaaacattcaaaaagaaattgaccgcctcaatgaggttgccaagaatttaaatgaatctctcatcgatctccaagaacttggaaagtat

SEQ ID NO: 11 - protein, 36 aa, synthetic construct
  source 1..36: note = Amino acid sequence of HR1-1
QKLIANQFNSAIGKIQDSLSSTASALGKLQDVVNQN

SEQ ID NO: 12 - protein, 42 aa, synthetic construct
  source 1..42: note = Amino acid sequence of HR1-2
KLIANQFNSAIGKIQDSLSSTASALGKLQDVVNQNAQALNTL

SEQ ID NO: 13 - protein, 40 aa, synthetic construct
  source 1..40: note = Amino acid sequence of HR1-3
ANQFNSAIGKIQDSLSSTASALGKLQDVVNQNAQALNTLV

SEQ ID NO: 14 - protein, 34 aa, synthetic construct
  source 1..34: note = Amino acid sequence of HR2-1
GINASVVNIQKEIDRLNEVAKNLNESLIDLQELG

SEQ ID NO: 15 - protein, 36 aa, synthetic construct
  source 1..36: note = Amino acid sequence of HR2-2
VDLGDISGINASVVNIQKEIDRLNEVAKNLNESLID

SEQ ID NO: 16 - protein, 36 aa, synthetic construct
  source 1..36: note = Amino acid sequence of HR2-3
DISGINASVVNIQKEIDRLNEVAKNLNESLIDLQEL

SEQ ID NO: 17 - DNA, 22 bp, synthetic construct
  source 1..22: mol_type = other DNA; note = SARS-CoV-2-NF
ggggaacttctcctgctagaat

SEQ ID NO: 18 - DNA, 22 bp, synthetic construct
  source 1..22: mol_type = other DNA; note = SARS-CoV-2-NR
cagacattttgctctcaagctg

SEQ ID NO: 19 - DNA, 20 bp, synthetic construct
  source 1..20: mol_type = other DNA; note = SARS-CoV-2-N-probe
ttgctgctgcttgacagatt

SEQ ID NO: 20 - DNA, 23 bp, synthetic construct
  source 1..23: mol_type = other DNA; note = SARS-CoV-2-EF
cgatctcttgtagatctgttctc

SEQ ID NO: 21 - DNA, 22 bp, synthetic construct
  source 1..22: mol_type = other DNA; note = SARS-CoV-2-ER
atattgcagcagtacgcacaca

SEQ ID NO: 22 - DNA, 26 bp, synthetic construct
  source 1..26: mol_type = other DNA; note = SARS-CoV-2-E-probe
cgaagcgcagtaaggatggctagtgt

SEQ ID NO: 23 - RNA, 633 nt, synthetic construct
  source 1..633: mol_type = other RNA; note = The mRNA sequence encoding HR121
atgacacagaatgttctctatgagaaccaaaaattgattgccaaccaatttaatagtgctattggcaaaattcaagactcactttcttccacagcaagtgcacttggaaaacttcaagatgtggtcaaccaaaatgcacaagctttaaacacgcttgttaaacaacttagctccaattttggtgcaatttcaagtgttttaaatgatatcctttcacgtcttgacaaagttgagggaggaagcggaggagatgttgatttaggtgacatctctggcattaatgcttcagttgtaaacattcaaaaagaaattgaccgcctcaatgaggttgccaagaatttaaatgaatctctcatcgatctccaagaacttggaaagtatagcggaggaagaggaggaacacagaatgttctctatgagaaccaaaaattgattgccaaccaatttaatagtgctattggcaaaattcaagactcactttcttccacagcaagtgcacttggaaaacttcaagatgtggtcaaccaaaatgcacaagctttaaacacgcttgttaaacaacttagctccaattttggtgcaatttcaagtgttttaaatgatatcctttcacgtcttgacaaagttgagtaa

SEQ ID NO: 24 - RNA, 357 nt, synthetic construct
  source 1..357: mol_type = other RNA; note = The mRNA sequence encoding HR121-1
atgcaaaaattgattgccaaccaatttaatagtgctattggcaaaattcaagactcactttcttccacagcaagtgcacttggaaaacttcaagatgtggtcaaccaaaatggaggaagcggaggaggcattaatgcttcagttgtaaacattcaaaaagaaattgaccgcctcaatgaggttgccaagaatttaaatgaatctctcatcgatctccaagaacttggaagcggaggaagaggaggacaaaaattgattgccaaccaatttaatagtgctattggcaaaattcaagactcactttcttccacagcaagtgcacttggaaaacttcaagatgtggtcaaccaaaattaa

SEQ ID NO: 25 - RNA, 399 nt, synthetic construct
  source 1..399: mol_type = other RNA; note = The mRNA sequence encoding HR121-2
atgaaattgattgccaaccaatttaatagtgctattggcaaaattcaagactcactttcttccacagcaagtgcacttggaaaacttcaagatgtggtcaaccaaaatgcacaagctttaaacacgcttggaggaagcggaggagttgatttaggtgacatctctggcattaatgcttcagttgtaaacattcaaaaagaaattgaccgcctcaatgaggttgccaagaatttaaatgaatctctcatcgatagcggaggaagaggaggaaaattgattgccaaccaatttaatagtgctattggcaaaattcaagactcactttcttccacagcaagtgcacttggaaaacttcaagatgtggtcaaccaaaatgcacaagctttaaacacgctttaa

SEQ ID NO: 26 - RNA, 399 nt, synthetic construct
  source 1..399: mol_type = other RNA; note = The mRNA sequence encoding HR123-1
atggccaaccaatttaatagtgctattggcaaaattcaagactcactttcttccacagcaagtgcacttggaaaacttcaagatgtggtcaaccaaaatgcacaagctttaaacacgcttgttaaacaaggaggaagcggaggagacatctctggcattaatgcttcagttgtaaacattcaaaaagaaattgaccgcctcaatgaggttgccaagaatttaaatgaatctctcatcgatctccaagaacttagcggaggaagaggaggagccaaccaatttaatagtgctattggcaaaattcaagactcactttcttccacagcaagtgcacttggaaaacttcaagatgtggtcaaccaaaatgcacaagctttaaacacgcttgttaaacaataa

SEQ ID NO: 27 - RNA, 534 nt, synthetic construct
  source 1..534: mol_type = other RNA; note = The mRNA sequence encoding HR212
atggatgttgatttaggtgacatctctggcattaatgcttcagttgtaaacattcaaaaagaaattgaccgcctcaatgaggttgccaagaatttaaatgaatctctcatcgatctccaagaacttggaaagtatagcggaggaagaggaggaacacagaatgttctctatgagaaccaaaaattgattgccaaccaatttaatagtgctattggcaaaattcaagactcactttcttccacagcaagtgcacttggaaaacttcaagatgtggtcaaccaaaatgcacaagctttaaacacgcttgttaaacaacttagctccaattttggtgcaatttcaagtgttttaaatgatatcctttcacgtcttgacaaagttgagggaggaagcggaggagatgttgatttaggtgacatctctggcattaatgcttcagttgtaaacattcaaaaagaaattgaccgcctcaatgaggttgccaagaatttaaatgaatctctcatcgatctccaagaacttggaaagtattaa

SEQ ID NO: 28 - RNA, 351 nt, synthetic construct
  source 1..351: mol_type = other RNA; note = The mRNA sequence encoding HR212-1
atgggcattaatgcttcagttgtaaacattcaaaaagaaattgaccgcctcaatgaggttgccaagaatttaaatgaatctctcatcgatctccaagaacttggaagcggaggaagaggaggacaaaaattgattgccaaccaatttaatagtgctattggcaaaattcaagactcactttcttccacagcaagtgcacttggaaaacttcaagatgtggtcaaccaaaatggaggaagcggaggaggcattaatgcttcagttgtaaacattcaaaaagaaattgaccgcctcaatgaggttgccaagaatttaaatgaatctctcatcgatctccaagaacttggataa

SEQ ID NO: 29 - RNA, 381 nt, synthetic construct
  source 1..381: mol_type = other RNA; note = The mRNA sequence encoding HR212-2
atggttgatttaggtgacatctctggcattaatgcttcagttgtaaacattcaaaaagaaattgaccgcctcaatgaggttgccaagaatttaaatgaatctctcatcgatagcggaggaagaggaggaaaattgattgccaaccaatttaatagtgctattggcaaaattcaagactcactttcttccacagcaagtgcacttggaaaacttcaagatgtggtcaaccaaaatgcacaagctttaaacacgcttggaggaagcggaggagttgatttaggtgacatctctggcattaatgcttcagttgtaaacattcaaaaagaaattgaccgcctcaatgaggttgccaagaatttaaatgaatctctcatcgattaa

SEQ ID NO: 30 - RNA, 381 nt, synthetic construct
  source 1..381: mol_type = other RNA; note = The mRNA sequence encoding HR212-3
atggacatctctggcattaatgcttcagttgtaaacattcaaaaagaaattgaccgcctcaatgaggttgccaagaatttaaatgaatctctcatcgatctccaagaacttagcggaggaagaggaggagccaaccaatttaatagtgctattggcaaaattcaagactcactttcttccacagcaagtgcacttggaaaacttcaagatgtggtcaaccaaaatgcacaagctttaaacacgcttgttaaacaaggaggaagcggaggagacatctctggcattaatgcttcagttgtaaacattcaaaaagaaattgaccgcctcaatgaggttgccaagaatttaaatgaatctctcatcgatctccaagaactttaa